European Patent Application EP 4 666 996 A1, published December 24, 2025. Title: Novel peptides with oral anti-aging properties. Applicant: QUIRIS Healthcare GmbH & Co. KGd, A.Costantino. The sequence listing filed with the application follows.

SEQUENCE LISTING (62 sequences)

SEQ ID NO: 1 - protein, 9 aa, Pisum sativum
ASDGSQEFK

SEQ ID NO: 2 - protein, 9 aa, Pisum sativum
DTSETWAIR

SEQ ID NO: 3 - protein, 9 aa, Pisum sativum
IFENLQNYR

SEQ ID NO: 4 - protein, 9 aa, Pisum sativum
LNQLDQVPR

SEQ ID NO: 5 - protein, 10 aa, Pisum sativum
DTMNINSLAR

SEQ ID NO: 6 - protein, 10 aa, Pisum sativum
FNLEEGDIMR

SEQ ID NO: 7 - protein, 10 aa, Pisum sativum
SDEEHQFESK

SEQ ID NO: 8 - protein, 10 aa, Pisum sativum
SSNTAGQIIK

SEQ ID NO: 9 - protein, 11 aa, Pisum sativum
GGLSIISPPEK

SEQ ID NO: 10 - protein, 11 aa, Pisum sativum
IDYGTNSMVNK

SEQ ID NO: 11 - protein, 11 aa, Pisum sativum
IQNAEDNVPQR

SEQ ID NO: 12 - protein, 11 aa, Pisum sativum
SSNNQLDQMPR

SEQ ID NO: 13 - protein, 12 aa, Pisum sativum
AKDTTMVDVPVK

SEQ ID NO: 14 - protein, 12 aa, Pisum sativum
GHEEIDKDETLK

SEQ ID NO: 15 - protein, 12 aa, Pisum sativum
LDEAAEPAALER

SEQ ID NO: 16 - protein, 12 aa, Pisum sativum
RQQGEETDAIVK

SEQ ID NO: 17 - protein, 12 aa, Pisum sativum
SRSDQENPFIFK

SEQ ID NO: 18 - protein, 17 aa, Pisum sativum
VTVTPGATDDQIMDGVR

SEQ ID NO: 19 - protein, 14 aa, Pisum sativum
DKRQQSQEENVIVK

SEQ ID NO: 20 - protein, 14 aa, Pisum sativum
DRRQEINEENVIVK

SEQ ID NO: 21 - protein, 10 aa, Pisum sativum
DTMNINSLAR

SEQ ID NO: 22 - protein, 9 aa, Pisum sativum
DTSETWAIR

SEQ ID NO: 23 - protein, 8 aa, Pisum sativum
DVVPEWVR

SEQ ID NO: 24 - protein, 8 aa, Pisum sativum
ENIADAAR

SEQ ID NO: 25 - protein, 12 aa, Pisum sativum
GHEEIDKDETLK

SEQ ID NO: 26 - protein, 17 aa, Pisum sativum
GSRQEEEEDEDEERQPR

SEQ ID NO: 27 - protein, 18 aa, Pisum sativum
KQKEGESEGEGEEAEVVK

SEQ ID NO: 28 - protein, 15 aa, Pisum sativum
LQGRNEDEEKGAIVK

SEQ ID NO: 29 - protein, 11 aa, Pisum sativum
NEDEEKGAIVK

SEQ ID NO: 30 - protein, 12 aa, Pisum sativum
PGLASTSGNISK

SEQ ID NO: 31 - protein, 11 aa, Pisum sativum
SSNNQLDQMPR

SEQ ID NO: 32 - protein, 11 aa, Pisum sativum
VSREQIEELSK

SEQ ID NO: 33 - protein, 17 aa, Pisum sativum
VTVTPGATDDQIMDGVR

SEQ ID NO: 34 - protein, 12 aa, Pisum sativum
LDEAAEPAALER

SEQ ID NO: 35 - protein, 8 aa, Pisum sativum
SVFNGEVR

SEQ ID NO: 36 - protein, 8 aa, Pisum sativum
EEELNNLR

SEQ ID NO: 37 - protein, 13 aa, Pisum sativum
EREEAEREQEAAR

SEQ ID NO: 38 - protein, 7 aa, Pisum sativum
HEIFQER

SEQ ID NO: 39 - protein, 22 aa, Pisum sativum
LKAEATSNYALSMSTHSQFISR

SEQ ID NO: 40 - protein, 7 aa, Pisum sativum
NRLELLK

SEQ ID NO: 41 - protein, 7 aa, Pisum sativum
SEPFNLR

SEQ ID NO: 42 - protein, 15 aa, Pisum sativum
GSRQEEDEDEEKQPR

SEQ ID NO: 43 - protein, 10 aa, Oryza sativa
AEDVGEEVER

SEQ ID NO: 44 - protein, 20 aa, Oryza sativa
AEPQPASPSAPGPTTDSEPK

SEQ ID NO: 45 - protein, 10 aa, Oryza sativa
AGFAGDDAPR

SEQ ID NO: 46 - protein, 21 aa, Oryza sativa
AGGEGDGEGKGGEGKGGHCCC

SEQ ID NO: 47 - protein, 23 aa, Oryza sativa
CSGETAAAVPAPVGTAVGSMGSR

SEQ ID NO: 48 - protein, 12 aa, Oryza sativa
DVVLLGATGTGK

SEQ ID NO: 49 - protein, 20 aa, Oryza sativa
EAWFAYLEAHPDLAPDFTER

SEQ ID NO: 50 - protein, 11 aa, Oryza sativa
GQIDDLLGEIR

SEQ ID NO: 51 - protein, 20 aa, Oryza sativa
HNVATPYHPQTSGQAETSNK

SEQ ID NO: 52 - protein, 21 aa, Oryza sativa
MTETRTHSAPWRNAAATPEER

SEQ ID NO: 53 - protein, 24 aa, Oryza sativa
SPVLVAIVGVVVLLVLLALVVVTR

SEQ ID NO: 54 - protein, 21 aa, Oryza sativa
YVELYAKDEDAFFRDYAESHK

SEQ ID NO: 55 - protein, 7 aa, Oryza sativa
ADTYNPR

SEQ ID NO: 56 - protein, 9 aa, Oryza sativa
ATPCGSGGR

SEQ ID NO: 57 - protein, 9 aa, Oryza sativa
AVFPSIVGR

SEQ ID NO: 58 - protein, 9 aa, Oryza sativa
GFQLGINLR

SEQ ID NO: 59 - protein, 10 aa, Oryza sativa
LVMLKAMDAR

SEQ ID NO: 60 - protein, 9 aa, Oryza sativa
SGSGGGGPR

SEQ ID NO: 61 - protein, 7 aa, Oryza sativa
STELLIR

SEQ ID NO: 62 - protein, 18 aa, Oryza sativa
VAPEEHPVLLTEAPLNPK